European Patent Application EP 4 289 946 A1, published December 13, 2023. Title: CONSTRUCTION AND APPLICATIONS OF ENATIOSELECTIVE FLIPPED ω-TRANSAMINASE MUTANT. Applicant: ZHEJIANG APELOA KANGYU PHARMACEUTICAL CO., LTD. APELOA PHARMACEUTICAL CO., LTD. The sequence listing filed with the application follows.

SEQUENCE LISTING (14 sequences)

SEQ ID NO: 1 - protein, 330 aa, Artificial Sequence
  ATA117_ACHH amino acid sequence
MAFSADTSEIVYTHDTGLDYITYSDYELDPANPLAGGAAWIEGAFVPPSEARISIFDQGYLHSDVTYTAFHVWNGNAFRLDDHIERLFSNAESMRIIPPLTQDEVKEIALELVAKTELREACVSVSITRGYSSTPGERDITKHRPQVYMYAVPYQWHVPFDRIRDGVHAMVAQSVRRTPRSSIDPQVKNFQWGDLIRAVQETHDRGFEAPLLLDGDGLLAEGSGHNVVVIKDGVVRSPGRAALPGITRKTVLEIAESLGHEAILADITLAELLDADEVLGCTTAGGVWPFVSVDGNPISDGVPGPVTQSIIRRYWELNVESSSLLTPVQY

SEQ ID NO: 2 - DNA, 993 bp, Artificial Sequence
  ATA117_ACHH nucleotide sequence
atggcatttagcgcggataccagcgaaatcgtctatacccacgataccggtctggattacatcacctacagcgattacgaactggatccggcaaatccgttagcaggcggcgcagcttggattgaaggcgcatttgttccgccgtctgaagcgcgtattagcatcttcgatcagggctatctgcatagcgacgttacctataccgcattccacgtttggaacggtaacgcatttcgtctggacgatcacatcgaacgtctgttcagcaacgccgaaagtatgcgtattattccgccgctgacccaagacgaagtcaaagaaatcgcgctggaactggttgcaaaaaccgaactgcgcgaagcgtgtgttagcgttagcattacccgcggttatagtagtaccccgggcgaacgcgatattaccaaacatcgtccgcaggtctacatgtacgctgttccgtaccagtggcatgttccgtttgatcgtattcgcgacggcgttcacgcaatggttgcacagagcgtgcgtcgtaccccgcgtagcagcatcgatccgcaggtcaaaaacttccagtggggcgatttaattcgcgcagttcaggaaacccacgatcgcggttttgaagcaccgttactgttagacggcgacggtttactggcagaaggtagcggccataacgtcgtcgtcattaaagatggggttgttcgttctccgggtcgtgcagcattaccgggtattacccgcaaaaccgttctggaaattgcggaatccctgggtcatgaagcgattctggcggatattaccttagcggaactgctggacgcagacgaagttttaggttgtaccaccgctggcggcgtttggccgtttgttagcgttgacggcaatccgattagcgatggtgttccgggtccggttacccaaagcattattcgtcgctactgggagctgaacgttgaaagtagcagcctgttaaccccggttcagtattaa

SEQ ID NO: 3 - DNA, 45 bp, Artificial Sequence
  VN-F
  misc_feature (19)..(19): n is a, c, g or t
  misc_feature (20)..(20): n is a, c, g or t
  misc_feature (21)..(21): k is t or g
agcgacgttacctataccnnkttccacgtttggaacggtaacgca

SEQ ID NO: 4 - DNA, 45 bp, Artificial Sequence
  VN-R
  misc_feature (19)..(19): m is a or c
  misc_feature (20)..(20): n is a, c, g or t
  misc_feature (21)..(21): n is a, c, g or t
accgttccaaacgtggaamnnggtataggtaacgtcgctatgcag

SEQ ID NO: 5 - DNA, 45 bp, Artificial Sequence
  FN-F
  misc_feature (19)..(19): n is a, c, g or t
  misc_feature (20)..(20): n is a, c, g or t
  misc_feature (21)..(21): k is t or g
accgaactgcgcgaagcgnnkgttagcgttagcattacccgcggt

SEQ ID NO: 6 - DNA, 45 bp, Artificial Sequence
  FN-R
  misc_feature (19)..(19): m is a or c
  misc_feature (20)..(20): n is a, c, g or t
  misc_feature (21)..(21): n is a, c, g or t
ggtaatgctaacgctaacmnncgcttcgcgcagttcggtttttgc

SEQ ID NO: 7 - DNA, 45 bp, Artificial Sequence
  IN-F
  misc_feature (19)..(19): n is a, c, g or t
  misc_feature (20)..(20): n is a, c, g or t
  misc_feature (21)..(21): k is t or g
gctgttccgtaccagtggnnkgttccgtttgatcgtattcgcgac

SEQ ID NO: 8 - DNA, 45 bp, Artificial Sequence
  IN-R
  misc_feature (19)..(19): m is a or c
  misc_feature (20)..(20): n is a, c, g or t
  misc_feature (21)..(21): n is a, c, g or t
aatacgatcaaacggaacmnnccactggtacggaacagcgtacat

SEQ ID NO: 9 - DNA, 45 bp, Artificial Sequence
  FN-F
  misc_feature (19)..(19): n is a, c, g or t
  misc_feature (20)..(20): n is a, c, g or t
  misc_feature (21)..(21): k is t or g
ctggcagaaggtagcggcnnkaacgtcgtcgtcattaaagatggg

SEQ ID NO: 10 - DNA, 45 bp, Artificial Sequence
  FN-R
  misc_feature (19)..(19): m is a or c
  misc_feature (20)..(20): n is a, c, g or t
  misc_feature (21)..(21): n is a, c, g or t
tttaatgacgacgacgttmnngccgctaccttctgccagtaaacc

SEQ ID NO: 11 - protein, 663 aa, Artificial Sequence
  Amino acid sequence of Escherichia coli transketolase
MSSRKELANAIRALSMDAVQKAKSGHPGAPMGMADIAEVLWRDFLKHNPQNPSWADRDRFVLSNGHGSMLIYSLLHLTGYDLPMEELKNFRQLHSKTPGHPEVGYTAGVETTTGPLGQGIANAVGMAIAEKTLAAQFNRPGHDIVDHYTYAFMGDGCMMEGISHEVCSLAGTLKLGKLIAFYDDNGISIDGHVEGWFTDDTAMRFEAYGWHVIRDIDGHDAASIKRAVEEARAVTDKPSLLMCKTIIGFGSPNKAGTHDSHGAPLGDAEIALTREQLGWKYAPFEIPSEIYAQWDAKEAGQAKESAWNEKFAAYAKAYPQEAAEFTRRMKGEMPSDFDAKAKEFIAKLQANPAKIASRKASQNAIEAFGPLLPEFLGGSADLAPYNLTLWSGSKAINEDAAGNYIHYGVREFGMTAIANGISLHGGFLPYTSTFLMFVEYARNAVRMAALMKQRQVMVYTHDSIGLGETGPTHQPVEQVASLRVTPNMSTWRPCDQVESAVAWKYGVERQDGPTALILSQQNLAQQERTEEQLANIARGGYVLKDCAGQPELIFIATGSEVELAVAAYEKLTAEGVKARVVSMPSTDAFDKQDAAYRESVLPKAVTARVAVEAGIADYWYKYVGLNGAIVGMTTFGESAPAELLFEEFGFTVDNVVAKAKELL

SEQ ID NO: 12 - DNA, 1992 bp, Artificial Sequence
  Nucleotide sequence of E. coli transketolase
atgtcctcacgtaaagagcttgccaatgctattcgtgcgctgagcatggacgcagtacagaaagccaaatccggtcacccgggtgcccctatgggtatggctgacattgccgaagtcctgtggcgtgatttcctgaaacacaacccgcagaatccgtcctgggctgaccgtgaccgcttcgtgctgtccaacggccacggctccatgctgatctacagcctgctgcacctcaccggttacgatctgccgatggaagaactgaaaaacttccgtcagctgcactctaaaactccgggtcacccggaagtgggttacaccgctggtgtggaaaccaccaccggtccgctgggtcagggtattgccaacgcagtcggtatggcgattgcagaaaaaacgctggcggcgcagtttaaccgtccgggccacgacattgtcgaccactacacctacgccttcatgggcgacggctgcatgatggaaggcatctcccacgaagtttgctctctggcgggtacgctgaagctgggtaaactgattgcattctacgatgacaacggtatttctatcgatggtcacgttgaaggctggttcaccgacgacaccgcaatgcgtttcgaagcttacggctggcacgttattcgcgacatcgacggtcatgacgcggcatctatcaaacgcgcagtagaagaagcgcgcgcagtgactgacaaaccttccctgctgatgtgcaaaaccatcatcggtttcggttccccgaacaaagccggtacccacgactcccacggtgcgccgctgggcgacgctgaaattgccctgacccgcgaacaactgggctggaaatatgcgccgttcgaaatcccgtctgaaatctatgctcagtgggatgcgaaagaagcaggccaggcgaaagaatccgcatggaacgagaaattcgctgcttacgcgaaagcttatccgcaggaagccgctgaatttacccgccgtatgaaaggcgaaatgccgtctgacttcgacgctaaagcgaaagagttcatcgctaaactgcaggctaatccggcgaaaatcgccagccgtaaagcgtctcagaatgctatcgaagcgttcggtccgctgttgccggaattcctcggcggttctgctgacctggcgccgtataacctgaccctgtggtctggttctaaagcaatcaacgaagatgctgcgggtaactacatccactacggtgttcgcgagttcggtatgaccgcgattgctaacggtatctccctgcacggtggcttcctgccgtacacctccaccttcctgatgttcgtggaatacgcacgtaacgccgtacgtatggctgcgctgatgaaacagcgtcaggtgatggtttacacccacgactccatcggtctgggcgaaaccggcccgactcaccagccggttgagcaggtcgcttctctgcgcgtaaccccgaacatgtctacatggcgtccgtgtgaccaggttgaatccgcggtcgcgtggaaatacggtgttgagcgtcaggacggcccgaccgcactgatcctctcccaacagaacctggcgcagcaggaacgaactgaagagcaactggcaaacatcgcgcgcggtggttatgtgctgaaagactgcgccggtcagccggaactgattttcatcgctaccggttcagaagttgaactggctgttgctgcctacgaaaaactgactgccgaaggcgtgaaagcgcgcgtggtgtccatgccgtctaccgacgcatttgacaagcaggatgctgcttaccgtgaatccgtactgccgaaagcggttactgcacgcgttgctgtagaagcgggtattgctgactactggtacaagtatgttggcctgaacggtgctatcgtcggtatgaccaccttcggtgaatctgctccggcagagctgctgtttgaagagttcggcttcactgttgataacgttgttgcgaaagcaaaagaactgctgtaa

SEQ ID NO: 13 - protein, 330 aa, Artificial Sequence
  Amino acid sequence of the transaminase ATA117
MAFSADTSEIVYTHDTGLDYITYSDYELDPANPLAGGAAWIEGAFVPPSEARISIFDQGYLHSDVTYTVFHVWNGNAFRLDDHIERLFSNAESMRIIPPLTQDEVKEIALELVAKTELREAFVSVSITRGYSSTPGERDITKHRPQVYMYAVPYQWIVPFDRIRDGVHAMVAQSVRRTPRSSIDPQVKNFQWGDLIRAVQETHDRGFEAPLLLDGDGLLAEGSGFNVVVIKDGVVRSPGRAALPGITRKTVLEIAESLGHEAILADITLAELLDADEVLGCTTAGGVWPFVSVDGNPISDGVPGPVTQSIIRRYWELNVESSSLLTPVQY

SEQ ID NO: 14 - DNA, 990 bp, Artificial Sequence
  Nucleotide sequence of the transaminase ATA117
atggcatttagcgcggataccagcgaaatcgtctatacccacgataccggtctggattacatcacctacagcgattacgaactggatccggcaaatccgttagcaggcggcgcagcttggattgaaggcgcatttgttccgccgtctgaagcgcgtattagcatcttcgatcagggctatctgcatagcgacgttacctataccgtcttccacgtttggaacggtaacgcatttcgtctggacgatcacatcgaacgtctgttcagcaacgccgaaagtatgcgtattattccgccgctgacccaagacgaagtcaaagaaatcgcgctggaactggttgcaaaaaccgaactgcgcgaagcgtttgttagcgttagcattacccgcggttatagtagtaccccgggcgaacgcgatattaccaaacatcgtccgcaggtctacatgtacgctgttccgtaccagtggatcgttccgtttgatcgtattcgcgacggcgttcacgcaatggttgcacagagcgtgcgtcgtaccccgcgtagcagcatcgatccgcaggtcaaaaacttccagtggggcgatttaattcgcgcagttcaggaaacccacgatcgcggttttgaagcaccgttactgttagacggcgacggtttactggcagaaggtagcggctttaacgtcgtcgtcattaaagatggggttgttcgttctccgggtcgtgcagcattaccgggtattacccgcaaaaccgttctggaaattgcggaatccctgggtcatgaagcgattctggcggatattaccttagcggaactgctggacgcagacgaagttttaggttgtaccaccgctggcggcgtttggccgtttgttagcgttgacggcaatccgattagcgatggtgttccgggtccggttacccaaagcattattcgtcgctactgggagctgaacgttgaaagtagcagcctgttaaccccggttcagtat